European Patent Application EP 4 282 488 A1, published November 29, 2023. Title: A method for evaluating an ability of test sample to activate xenobiotic response in the skin, a method for screening a substance having an ability to suppress xenobiotic response in the skin, and an agent for supressing xenobiotic response in the skin. Applicant: NATIONAL UNIVERSITY CORPORATION KOBE UNIVERSITY NATIONAL UNIVERSITY CORPORATION OKAYAMA UNIVRESITY. The sequence listing filed with the application follows.

SEQUENCE LISTING (10 sequences)

SEQ ID NO: 1 - DNA, 19 bp, Artificial
  Foward PCR primer for GAPDH
agccacatcgctcagacac

SEQ ID NO: 2 - DNA, 19 bp, Artificial
  Reverse PCR primer for GAPDH
gcccaatacgaccaaatcc

SEQ ID NO: 3 - DNA, 21 bp, Artificial
  Forward PCR primer for Artemin
cgctcctggtgttgatagaga

SEQ ID NO: 4 - DNA, 18 bp, Artificial
  Reverse PCR primer for Artemin
gcggagagaccaagtgga

SEQ ID NO: 5 - DNA, 20 bp, Artificial
  Forward PCR primer for MMP9
gaaccaatctcaccgacagg

SEQ ID NO: 6 - DNA, 20 bp, Artificial
  Reverse PCR primer for MMP9
gccacccgagtgtaaccata

SEQ ID NO: 7 - DNA, 22 bp, Artificial
  Foward PCR primer for MMP2
agcgagtggatgccgcctttaa

SEQ ID NO: 8 - DNA, 22 bp, Artificial
  Reverse PCR primer for MMP2
cattccaggcatctgcgatgag

SEQ ID NO: 9 - DNA, 24 bp, Artificial
  Forward PCR primer for TIMP-1
aagacctacactgttggctgtgag

SEQ ID NO: 10 - DNA, 20 bp, Artificial
  Reverse PCR primer for TIMP-1
gtccgtccacaagcaatgag